European Patent Application EP 4 609 881 A1, published September 3, 2025. Title: Radioactive pharmaceutical composition. Applicant: 日本メジフィジックス株式会社. The sequence listing filed with the application follows.

SEQUENCE LISTING (24 sequences)

SEQ ID NO: 1 - protein, 121 aa, synthetic construct
  REGION 1..121: note = Humanaized antibody heavy chain variable region 1 (H01)
EVQLLESGGGLVQPGGSLRLSCAASGFTFSNYGMSWVRQAPGKGLEWVSTISNSGRYTYFPDSVKGRFTISRDNSKNTLYLQMNSLRAEDTALYYCTRHLDYANYDAMDYWGQGTLVTVSS

SEQ ID NO: 2 - protein, 121 aa, synthetic construct
  REGION 1..121: note = Humanaized antibody heavy chain variable region 2 (H02)
LVQLVESGGGVVRPGGSLRLSCAASGFTFSNYGMSWIRQAPGKGLEWVSTISNSGRYTYFPDSVKGRFTISRDNAKNSLYLQMNSLRAEDTALYYCTRHLDYANYDAMDYWGQGTLVTVSS

SEQ ID NO: 3 - protein, 121 aa, synthetic construct
  REGION 1..121: note = Humanaized antibody heavy chain variable region 3 (H03)
LVQLVESGGGVVQPGRSLRLSCAASGFTFSNYGMSWVRQAPGKGLEWVATISNSGRYTYFPDSVKGRFTISRDNSKNTLYLQMNSLRAEDTAVYYCTRHLDYANYDAMDYWGQGTLVTVSS

SEQ ID NO: 4 - protein, 121 aa, synthetic construct
  REGION 1..121: note = Humanaized antibody heavy chain variable region 4 (H04)
EVQLLESGGGLVQPGGSLRLSCAVSGFTFSNYGMSWVRQAPGKGLEWVSTISNSGRYTYFPDSVKGRFTISRDNSRNTLYLQMNTLRAEDTAVYYCTRHLDYANYDAMDYWGQGTPVTVSS

SEQ ID NO: 5 - protein, 111 aa, synthetic construct
  REGION 1..111: note = Humanaized antibody light chain variable region 1 (L01)
DIVMTQSPSSLSASVGDRVTITCRASKSVTTSDFSYMHWYQQKPGKAPKLLIYLASNLESGVPSRFSGSGSGTDFTLTISSLQPEDFATYYCQHSREFPWTFGGGTKVEIK

SEQ ID NO: 6 - protein, 111 aa, synthetic construct
  REGION 1..111: note = Humanaized antibody light chain variable region 2 (L02)
DVVMTQSPSTLSASVGDRVTITCRASKSVTTSDFSYMHWYQQKPGQAPKLLIYLASNLESGVPSRFSGSGSGTDFTLTISSLQPEDFATYYCQHSREFPWTFGQGTKLEIK

SEQ ID NO: 7 - protein, 111 aa, synthetic construct
  REGION 1..111: note = Humanaized antibody light chain variable region 3 (L03)
DIQMTQSPSSLSASVGDRVTITCRASKSVTTSDFSYMHWYQQKPGKSPKLLIYLASNLESGVPSRFSGSGSGTDFSLTISSLQPEDFATYYCQHSREFPWTFGGGTKVEIK

SEQ ID NO: 8 - protein, 111 aa, synthetic construct
  REGION 1..111: note = Humanaized antibody light chain variable region 4 (L04)
DIVMTQSPDSLAVSLGERATINCKASKSVTTSDFSYLHWYQQKPGQPPKLLIYLASNLESGVPDRFSGSGSGTDFTLTISSLQAEDVAVYYCQHSREFPWTFGGGTKLEIK

SEQ ID NO: 9 - protein, 13 aa, synthetic construct
  REGION 1..13: note = antibody modifying peptide
  SITE 6: note = misc_feature - lysine, cystein, aspartic acid, glutamic acid, 2-aminosuberic acid, or diaminopropionic acid
DCAYHXGELVWCT

SEQ ID NO: 10 - protein, 17 aa, synthetic construct
  REGION 1..17: note = antibody modifying peptide
  SITE 8: note = misc_feature - lysine, cystein, aspartic acid, glutamic acid, 2-aminosuberic acid, or diaminopropionic acid
GPDCAYHXGELVWCTFH

SEQ ID NO: 11 - protein, 13 aa, synthetic construct
  REGION 1..13: note = antibody modifying peptide
  SITE 6: note = misc_feature - lysine, cystein, aspartic acid, glutamic acid, 2-aminosuberic acid, or diaminopropionic acid
RCAYHXGELVWCS

SEQ ID NO: 12 - protein, 17 aa, synthetic construct
  REGION 1..17: note = antibody modifying peptide
  SITE 8: note = misc_feature - lysine, cystein, aspartic acid, glutamic acid, 2-aminosuberic acid, or diaminopropionic acid
GPRCAYHXGELVWCSFH

SEQ ID NO: 13 - protein, 17 aa, synthetic construct
  REGION 1..17: note = antibody modifying peptide
  SITE 8: note = misc_feature - lysine, cystein, aspartic acid, glutamic acid, 2-aminosuberic acid, or diaminopropionic acid
SPDCAYHXGELVWCTFH

SEQ ID NO: 14 - protein, 17 aa, synthetic construct
  REGION 1..17: note = antibody modifying peptide
  SITE 8: note = misc_feature -lysine, cystein, aspartic acid, glutamic acid, 2-aminosuberic acid, or diaminopropionic acid
GDDCAYHXGELVWCTFH

SEQ ID NO: 15 - protein, 17 aa, synthetic construct
  REGION 1..17: note = antibody modifying peptide
  SITE 8: note = misc_feature - lysine, cystein, aspartic acid, glutamic acid, 2-aminosuberic acid, or diaminopropionic acid
GPSCAYHXGELVWCTFH

SEQ ID NO: 16 - protein, 17 aa, synthetic construct
  REGION 1..17: note = antibody modifying peptide
  SITE 8: note = misc_feature - lysine, cystein, aspartic acid, glutamic acid, 2-aminosuberic acid, or diaminopropionic acid
GPDCAYHXGELVWCSFH

SEQ ID NO: 17 - protein, 17 aa, synthetic construct
  REGION 1..17: note = antibody modifying peptide
  SITE 8: note = misc_feature - lysine, cystein, aspartic acid, glutamic acid, 2-aminosuberic acid, or diaminopropionic acid
GPDCAYHXGELVWCTHH

SEQ ID NO: 18 - protein, 17 aa, synthetic construct
  REGION 1..17: note = antibody modifying peptide
  SITE 8: note = misc_feature - lysine, cystein, aspartic acid, glutamic acid, 2-aminosuberic acid, or diaminopropionic acid
GPDCAYHXGELVWCTFY

SEQ ID NO: 19 - protein, 17 aa, synthetic construct
  REGION 1..17: note = antibody modifying peptide
  SITE 8: note = misc_feature -lysine, cystein, aspartic acid, glutamic acid, 2-aminosuberic acid, or diaminopropionic acid
SPDCAYHXGELVWCTFY

SEQ ID NO: 20 - protein, 17 aa, synthetic construct
  REGION 1..17: note = antibody modifying peptide
  SITE 8: note = misc_feature - lysine, cystein, aspartic acid, glutamic acid, 2-aminosuberic acid, or diaminopropionic acid
SDDCAYHXGELVWCTFY

SEQ ID NO: 21 - protein, 17 aa, synthetic construct
  REGION 1..17: note = antibody modifying peptide
  SITE 8: note = misc_feature - lysine, cystein, aspartic acid, glutamic acid, 2-aminosuberic acid, or diaminopropionic acid
RGNCAYHXGQLVWCTYH

SEQ ID NO: 22 - protein, 17 aa, synthetic construct
  REGION 1..17: note = antibody modifying peptide
  SITE 2: note = misc_feature - homocysteine
  SITE 8: note = misc_feature - lysine, cystein, aspartic acid, glutamic acid, 2-aminosuberic acid, or diaminopropionic acid
  SITE 16: note = misc_feature - homocysteine
GXDCAYHXGELVWCTXH

SEQ ID NO: 23 - protein, 330 aa, synthetic construct [sequence omitted]

SEQ ID NO: 24 - protein, 107 aa, synthetic construct [sequence omitted]